European Patent Specification EP 3 819 390 B1, published October 18, 2023. Title: RAPID AMPLIFICATION METHOD FOR NUCLEIC ACID OF HEPATITIS B VIRUS. Applicant: SANSURE BIOTECH INC. Application EP19830704.3. The sequence listing filed with the application follows.

SEQUENCE LISTING (5 sequences)

SEQ ID NO: 1 - DNA, 26 bp, Artificial Sequence
  Hepatitis B virus - forward primer
atcgctggatgtgtctgctgcgtttt

SEQ ID NO: 2 - DNA, 28 bp, Artificial Sequence
  Hepatitis B virus - reverse primer
ctggaattagaggacaaacgggcaacat

SEQ ID NO: 3 - DNA, 38 bp, Artificial Sequence
  first probe
cctcttcatcctgctgctatgcctcatcttcttattgg

SEQ ID NO: 4 - DNA, 97 bp, Artificial Sequence
  Hepatitis B virus - sequence for forming internal standard
atcgctggatgtgtctgcggcgttttatatcttcctccatcctgctaggtgcctcatcttcttagctctatgttgcccgtttgtcctctaattccag

SEQ ID NO: 5 - DNA, 36 bp, Artificial Sequence
  second probe
ttcctccatcctgctaggtgcctcatcttcttagct